European Patent Application EP 4 289 958 A1, published December 13, 2023. Title: Proteins with 1,3-fucosyltransferase activity and Method for producing fucose-containing carbohydrates. Applicant: KYOWA HAKKO BIO CO., LTD. The sequence listing filed with the application follows.

SEQUENCE LISTING (39 sequences)

SEQ ID NO: 1 - DNA, 951 bp, Bacteroides reticulotermitis
atgaaattgaaagtgaaatttgtagatttttgggatggctttgatgaacattataatactttcgttaatgttctatctgagaaatatgaaatcgaaatttgtgatcatcctgattacttaatatattcgacttttggatataagaacttaaagtacgaaaattgtgttaagatattttatacgggtgaaaatataactccagactttaatctttgtgattatgcgattggctttgatataatggaattcggagatcgctatatgcgcctaccattatatgccttatatggtattgaagagttgcgtaaacctaaagtctttaattcacaggaagctctgaatcggaaattctgtagttttgttgtctctaatggagctgatgctcctgaaaggacccgtttctttcatttactttcagaatataagcaggtagattcaggaggagcatatgagaataatgttggtgggcgagttgttgataagaaattttttatttctaactataaattcaatattgcttttgaaaatagtgctaaagacggatatactacagagaaaattatggagccgatgttggtaaactctctgccgatatattggggaaacagattggttgagttggattttaatcctaattcttttattaatgctgcagattacccatctttagaagctttggtagaatatatcgttgagttggacacaaatgatgataaatatctgtcaattttgtcaagaccttggcttaacaaaagtaattatttggattggcaagaaaggctttttagcttctttgagaatgttttcaataaaccattgaatgaacagaaatatttatcaccttatgggtacggtaagctatatagaagaagattaatggaaatgtatattgcgaaaagaaaattgaaaaaatggaaaatggtttgtaacccttgtcgttggtttagatga

SEQ ID NO: 2 - protein, 316 aa, Bacteroides reticulotermitis
MKLKVKFVDFWDGFDEHYNTFVNVLSEKYEIEICDHPDYLIYSTFGYKNLKYENCVKIFYTGENITPDFNLCDYAIGFDIMEFGDRYMRLPLYALYGIEELRKPKVFNSQEALNRKFCSFVVSNGADAPERTRFFHLLSEYKQVDSGGAYENNVGGRVVDKKFFISNYKFNIAFENSAKDGYTTEKIMEPMLVNSLPIYWGNRLVELDFNPNSFINAADYPSLEALVEYIVELDTNDDKYLSILSRPWLNKSNYLDWQERLFSFFENVFNKPLNEQKYLSPYGYGKLYRRRLMEMYIAKRKLKKWKMVCNPCRWFR

SEQ ID NO: 3 - DNA, 954 bp, Bacteroides reticuloterimis and Bacteroides fragilis
atgaaattgaaagtgaaatttgtagatttttgggatggctttgatgaacattataatactttcgttaatgttctatctgagaaatatgaaatcgaaatttgtgatcatcctgattacttaatatattcgacttttggatataagaacttaaagtacgaaaattgtgttaagatattttatacgggtgaaaatataactccagactttaatctttgtgattatgcgattggctttgatataatggaattcggagatcgctatatgcgcctaccattatatgccttatatggtattgaagagttgcgtaaacctaaagtctttaattcacaggaagctctgaatcgtaagttctgcagcatcgtggttagcaataataaatgggcggacccgattcgtgagacctttttcaaactgctgagcagctacaaaaaggtggacagcggtggccgtgcgtggaacaacatcggtggcccggttgacaacaagctggatttcatcagccagtacaaattcaacattgcgtttgagaacagccgtgtgctgggttacaccaccgaaaagattatggagccgatgcaagtgaacagcattccggtttactggggtaacagattggttgagttggattttaatcctaattcttttattaatgctgcagattacccatctttagaagctttggtagaatatatcgttgagttggacacaaatgatgataaatatctgtcaattttgtcaagaccttggcttaacaaaagtaattatttggattggcaagaaaggctttttagcttctttgagaatgttttcaataaaccattgaatgaacagaaatatttatcaccttatgggtacggtaagctatatagaagaagattaatggaaatgtatattgcgaaaagaaaattgaaaaaatggaaaatggtttgtaacccttgtcgttggtttagatga

SEQ ID NO: 4 - protein, 317 aa, Bacteroides reticuloterimis and Bacteroides fragilis
MKLKVKFVDFWDGFDEHYNTFVNVLSEKYEIEICDHPDYLIYSTFGYKNLKYENCVKIFYTGENITPDFNLCDYAIGFDIMEFGDRYMRLPLYALYGIEELRKPKVFNSQEALNRKFCSIVVSNNKWADPIRETFFKLLSSYKKVDSGGRAWNNIGGPVDNKLDFISQYKFNIAFENSRVLGYTTEKIMEPMQVNSIPVYWGNRLVELDFNPNSFINAADYPSLEALVEYIVELDTNDDKYLSILSRPWLNKSNYLDWQERLFSFFENVFNKPLNEQKYLSPYGYGKLYRRRLMEMYIAKRKLKKWKMVCNPCRWFR

SEQ ID NO: 5 - DNA, 996 bp, Bacteroides fragilis
atgtgtgattgcttgtctatcatattgttagtcaaaatgaaaaagatttatttgaaatttgttgatttttgggatggatttgatactatttctaactttattgtggatgctttgtccattcaatacgaagtagtactatctaatgagccagattatttattctattcatgttttggaacgtcacatttagaatatgattgtataaaaatcatgtttataggtgaaaatatagttcctgattttaacgtttgtgattatgccataggttttaattatattgattttggggaccgttacttgaggttgcctttatatgctatatatgatggattttcaaacttgcagaataaaaagattgatgtaaataaagctttagaccgtaaattttgtagtattgttgtttcaaataataaatgggcagatcctattcgtgagactttctttaaattactatctagttataagaaagtagactctggtggaagagcttggaataatataggaggacctgttgataataaattggattttattagccaatataagtttaatattgcttttgaaaatagtagggtactgggatatacaacagaaaaaataatggaacctatgcaggtgaattctattccagtatattggggaaatcctttggttggtaaagattttaatgtggactcctttgtaaatgctcatgattttgattctttagaaagattagttgagtatattatagaattggattcttcaaaggataaatatctggaaatgttggaaaaaccttggcttctcgataagacatatttggattggaaacaattgctgttaaattttattaataatattatgatgaaatcatataaggatgcgaagtatttggttaattatggtcatgctggaaagtatagaaatgaacaacgcttttgggggagatgtgaacgtaaatttaaacttcaaagaattattgaatattattctcaattgtttgatagaaaataa

SEQ ID NO: 6 - protein, 331 aa, Bacteroides fragilis
MCDCLSIILLVKMKKIYLKFVDFWDGFDTISNFIVDALSIQYEVVLSNEPDYLFYSCFGTSHLEYDCIKIMFIGENIVPDFNVCDYAIGFNYIDFGDRYLRLPLYAIYDGFSNLQNKKIDVNKALDRKFCSIVVSNNKWADPIRETFFKLLSSYKKVDSGGRAWNNIGGPVDNKLDFISQYKFNIAFENSRVLGYTTEKIMEPMQVNSIPVYWGNPLVGKDFNVDSFVNAHDFDSLERLVEYIIELDSSKDKYLEMLEKPWLLDKTYLDWKQLLLNFINNIMMKSYKDAKYLVNYGHAGKYRNEQRFWGRCERKFKLQRIIEYYSQLFDRK

SEQ ID NO: 7 - DNA, 264 bp, Artificial Sequence
  Description of the artificial sequence: partial base sequence of codon-optimized BfFucT
cgtaagttctgcagcatcgtggttagcaataataaatgggcggacccgattcgtgagacctttttcaaactgctgagcagctacaaaaaggtggacagcggtggccgtgcgtggaacaacatcggtggcccggttgacaacaagctggatttcatcagccagtacaaattcaacattgcgtttgagaacagccgtgtgctgggttacaccaccgaaaagattatggagccgatgcaagtgaacagcattccggtttactggggt

SEQ ID NO: 8 - DNA, 20 bp, Artificial Sequence
  Description of the artificial sequence: base sequence of primer for amplification of cat
accaggcgtttaagggcacc

SEQ ID NO: 9 - DNA, 45 bp, Artificial Sequence
  Description of the artificial sequence: base sequence of primer for amplification of cat
gactacgggcctaaagtcgacagaataaataaatcctggtgtccc

SEQ ID NO: 10 - DNA, 28 bp, Artificial Sequence
  Description of the artificial sequence: base sequence of  primer for amplification of sacB
gtcgactttaggcccgtagtctgcaaat

SEQ ID NO: 11 - DNA, 21 bp, Artificial Sequence
  Description of the artificial sequence: base sequence of  primer for amplification of sacB
tacggttagccatttgcctgc

SEQ ID NO: 12 - DNA, 42 bp, Artificial Sequence
  Description of the artificial sequence: base sequence of primer for amplification of lacZ Upstream 1
ggtgcccttaaacgcctggtagctgtttcctgtgtgaaattg

SEQ ID NO: 13 - DNA, 18 bp, Artificial Sequence
  Description of the artificial sequence: base sequence of primer for amplification of lacZ Upstream 1
ccagtctggccctgcacg

SEQ ID NO: 14 - DNA, 43 bp, Artificial Sequence
  Description of the artificial sequence: base sequence of primer for  amplification of lacY Downstream 1
gcaggcaaatggctaaccgtacgaccaacatatcataacggag

SEQ ID NO: 15 - DNA, 20 bp, Artificial Sequence
  Description of the artificial sequence: base sequence of primer for  amplification of lacY Downstream 1
gtttccgctctgtttgctgc

SEQ ID NO: 16 - DNA, 42 bp, Artificial Sequence
  Description of the artificial sequence: base sequence of  primer for amplification of  lacZ Upstream 2
ccgttatgatatgttggtcgagctgtttcctgtgtgaaattg

SEQ ID NO: 17 - DNA, 22 bp, Artificial Sequence
  Description of the artificial sequence: base sequence of amplification primer for amplification of lacY Downstream 2
cgaccaacatatcataacggag

SEQ ID NO: 18 - DNA, 41 bp, Artificial Sequence
  Description of the artificial sequence: base sequence of primer for amplification of wcaJ Upstream 1
ggtgcccttaaacgcctggtcgttgttcctgttattagccc

SEQ ID NO: 19 - DNA, 20 bp, Artificial Sequence
  Description of the artificial sequence: base sequence of primer for amplification of wcaJ Upstream 1
acgcggtcgctatcagcaaa

SEQ ID NO: 20 - DNA, 44 bp, Artificial Sequence
  Description of the artificial sequence: base sequence of primer for amplification of wcaM Downstream 1
gcaggcaaatggctaaccgtaatttgcgaccattcctggaaaaa

SEQ ID NO: 21 - DNA, 23 bp, Artificial Sequence
  Description of the artificial sequence: base sequence of primer for amplification of wcaM Downstream 1
acttcacaaacgcctgcatatag

SEQ ID NO: 22 - DNA, 41 bp, Artificial Sequence
  Description of the artificial sequence: base sequence of primer for amplification of wcaJ Upstream 2
ttccaggaatggtcgcaaatcgttgttcctgttattagccc

SEQ ID NO: 23 - DNA, 23 bp, Artificial Sequence
  Description of the artificial sequence: base sequence of primer for amplification of wcaM Downstream 2
atttgcgaccattcctggaaaaa

SEQ ID NO: 24 - DNA, 26 bp, Artificial Sequence
  Description of the artificial sequence: base sequence of primer for amplification of rcsA
atgtcaacgattattatggatttatg

SEQ ID NO: 25 - DNA, 42 bp, Artificial Sequence
  Description of the artificial sequence: base sequence of primer for amplification of rcsA
cattctagacctccttaattagcgcatgttgacaaaaatacc

SEQ ID NO: 26 - DNA, 36 bp, Artificial Sequence
  Description of the artificial sequence: base sequence of primer for amplification of bffucT
aggaggtctagaatgtgtgattgcttgtctatcata

SEQ ID NO: 27 - DNA, 38 bp, Artificial Sequence
  Description of the artificial sequence: base sequence of primer for amplification of bffucT
ggatttcctctcgagttattttctatcaaacaattgag

SEQ ID NO: 28 - DNA, 38 bp, Artificial Sequence
  Description of the artificial sequence: base sequence of primer for amplification of brfucT
aggaggtctagaatgaaattgaaagtgaaatttgtaga

SEQ ID NO: 29 - DNA, 35 bp, Artificial Sequence
  Description of the artificial sequence: base sequence of primer for amplification of brfucT
ggatttcctctcgagtcatctaaaccaacgacaag

SEQ ID NO: 30 - DNA, 22 bp, Artificial Sequence
  Description of the artificial sequence: base sequence of primer for amplification of cBrFucT Upstream
attcagagcttcctgtgaatta

SEQ ID NO: 31 - DNA, 41 bp, Artificial Sequence
  Description of the artificial sequence: base sequence of primer for amplification of cBrFucT Midstream
attcacaggaagctctgaatcgtaagttctgcagcatcgtg

SEQ ID NO: 32 - DNA, 20 bp, Artificial Sequence
  Description of the artificial sequence: base sequence of primer for amplification of cBrFucT Midstream
accccagtaaaccggaatgc

SEQ ID NO: 33 - DNA, 40 bp, Artificial Sequence
  Description of the artificial sequence: base sequence of primer for amplification of cBrFucT Downstream
gcattccggtttactggggtaacagattggttgagttgga

SEQ ID NO: 34 - DNA, 45 bp, Artificial Sequence
  Description of the artificial sequence: base sequence of primer for amplification of lacY
ctcgagaggaaatccattatgtactatttaaaaaacacaaacttt

SEQ ID NO: 35 - DNA, 23 bp, Artificial Sequence
  Description of the artificial sequence: base sequence of primer for amplification of lacY
ttaagcgacttcattcacctgac

SEQ ID NO: 36 - DNA, 41 bp, Artificial Sequence
  Description of the artificial sequence: base sequence of primer for amplification of rcsA-cBrFucT-lacY
gaggagaaattaaccatgtcaacgattattatggatttatg

SEQ ID NO: 37 - DNA, 38 bp, Artificial Sequence
  Description of the artificial sequence: base sequence of primer for amplification of rcsA-cBrFucT-lacY
agggcatcggtcgacttaagcgacttcattcacctgac

SEQ ID NO: 38 - DNA, 21 bp, Artificial Sequence
  Description of the artificial sequence: base sequence of primer for amplification of pPE167
gtcgaccgatgcccttgagag

SEQ ID NO: 39 - DNA, 25 bp, Artificial Sequence
  Description of the artificial sequence: base sequence of primer for amplification of pPE167
ggttaatttctcctctttaatatcg